European Patent Specification EP 3 705 133 B1, published June 26, 2024. Title: CHIMERIC OSPA GENES AND METHODS OF USE THEREOF. Applicant: CROWE, et al. The sequence listing filed with the application follows.

SEQUENCE LISTING (173 sequences)

SEQ ID NO: 1 - DNA, 829 bp, Artificial Sequence
  Synthetic nucleotide
catatgcgtctgttgatcggctttgctctggcgctggctctgatcggctgcgcacagaaaggtgctgagtctattggttccgtttctgtagatctgcccggtgaaatgaaggttctggtgagcaaagaaaaagacaagaacggcaagtacgatctcatcgcaaccgtcgacaagctggagctgaaaggtacttctgataaaaacaacggctctggtgtgctggagggcgtcaaaactaacaagagcaaagtaaagcttacgatctctgacgatctcggtcagaccacgctggaagttttcaaagaggatggcaagaccctcgtgtccaaaaaagtaacttccaaagacaagtcctctacggaagaaaaattcaacgaaaaaggtgaggtgtctgaaaagatcatcaccatggcagacggcacccgtcttgaatacaccggtattaaaagcgatggtaccggtaaagcgaaatatgttctgaaaaacttcactctggaaggcaaagtggctaatgataaaaccaccttggaagtcaaggaaggcaccgttactctgagcatgaatatctccaaatctggtgaagtttccgttgaactgaacgacactgacagcagcgctgcgactaaaaaaactgcagcgtggaattccaaaacttctactttaaccattagcgttaacagcaaaaaaactacccagctggtgttcactaaacaagacacgatcactgtgcagaaatacgactccgcaggcaccaacttagaaggcacggcagtcgaaattaaaacccttgatgaactgaaaaacgcgctgaaataagctgagcggatcc

SEQ ID NO: 2 - protein, 270 aa, Artificial Sequence
  Synthetic peptide
MRLLIGFALALALIGCAQKGAESIGSVSVDLPGEMKVLVSKEKDKNGKYDLIATVDKLELKGTSDKNNGSGVLEGVKTNKSKVKLTISDDLGQTTLEVFKEDGKTLVSKKVTSKDKSSTEEKFNEKGEVSEKIITMADGTRLEYTGIKSDGTGKAKYVLKNFTLEGKVANDKTTLEVKEGTVTLSMNISKSGEVSVELNDTDSSAATKKTAAWNSKTSTLTISVNSKKTTQLVFTKQDTITVQKYDSAGTNLEGTAVEIKTLDELKNALK

SEQ ID NO: 3 - DNA, 832 bp, Artificial Sequence
  Synthetic nucleotide
catatgcgtctgttgatcggctttgctctggcgctggctctgatcggctgcgcacagaaaggtgctgagtctattggttccgtttctgtagatctgcccggtggcatgaccgttctggtcagcaaagaaaaagacaaaaacggtaaatacagcctcgaggcgaccgtcgacaagcttgagctgaaaggcacctctgataaaaacaacggttccggcaccctggaaggtgaaaaaactaacaaaagcaaagtgaaactgaccattgctgatgacctcagccagaccaaattcgaaattttcaaagaagatgccaaaaccttagtatccaaaaaagtgaccctgaaagacaagtcctctaccgaagaaaaattcaacgaaaagggtgaaacctctgaaaaaaccatcgtaatggcaaatggtacccgtctggaatacaccgacatcaaaagcgatggctccggcaaagccaaatacgttctgaaagacttcaccctggaaggcaccctcgctgccgacggcaaaaccaccttgaaagttaccgaaggcactgttgttttaagcatgaacatcttaaaatccggtgaaatcaccgttgcgctggatgactctgacaccactcaggccactaaaaaaaccggcaaatgggattctaacacttccactctgaccatcagcgtgaattccaaaaaaactaaaaacatcgtgttcaccaaagaagacaccatcaccgtccagaaatacgactctgcgggcaccaacctcgaaggcaacgcagtcgaaatcaaaaccctggatgaactgaaaaacgctctgaaataagctgagcggatcc

SEQ ID NO: 4 - protein, 271 aa, Artificial Sequence
  Synthetic peptide
MRLLIGFALALALIGCAQKGAESIGSVSVDLPGGMTVLVSKEKDKNGKYSLEATVDKLELKGTSDKNNGSGTLEGEKTNKSKVKLTIADDLSQTKFEIFKEDAKTLVSKKVTLKDKSSTEEKFNEKGETSEKTIVMANGTRLEYTDIKSDGSGKAKYVLKDFTLEGTLAADGKTTLKVTEGTVVLSMNILKSGEITVALDDSDTTQATKKTGKWDSNTSTLTISVNSKKTKNIVFTKEDTITVQKYDSAGTNLEGNAVEIKTLDELKNALK

SEQ ID NO: 5 - DNA, 829 bp, Artificial Sequence
  Synthetic nucleotide
catatgcgtctgttgatcggctttgctttggcgctggctttaatcggctgtgcacagaaaggtgctgagtctattggttccgtttctgtagatctgcccgggggtatgaaagttctggtaagcaaagaaaaagacaaaaacggtaaatacagcctgatggcaaccgtagaaaagctggagcttaaaggcacttctgataaaaacaacggttctggcaccctggaaggtgaaaaaactaacaaaagcaaagtaaagcttactattgctgaggatctgagcaaaaccacctttgaaatcttcaaagaagatggcaaaactctggtatctaaaaaagtaaccctgaaagacaagtcttctaccgaagaaaaattcaacgaaaagggtgaaatctctgaaaaaactatcgtaatggcaaatggtacccgtctggaatacaccgacatcaaaagcgataaaaccggcaaagctaaatacgttctgaaagactttactctggaaggcactctggctgctgacggcaaaaccactctgaaagttaccgaaggcactgttactctgagcatgaacatttctaaatccggcgaaatcaccgttgcactggatgacactgactctagcggcaataaaaaatccggcacctgggattctgatacttctactttaaccattagcaaaaacagccagaaaactaaacagctggtattcaccaaagaaaacactatcaccgtacagaactataaccgtgcaggcaatgcgctggaaggcagcccggctgaaattaaagatctggcagagctgaaagccgctttgaaataagctgagcggatcc

SEQ ID NO: 6 - protein, 270 aa, Artificial Sequence
  Synthetic peptide
MRLLIGFALALALIGCAQKGAESIGSVSVDLPGGMKVLVSKEKDKNGKYSLMATVEKLELKGTSDKNNGSGTLEGEKTNKSKVKLTIAEDLSKTTFEIFKEDGKTLVSKKVTLKDKSSTEEKFNEKGEISEKTIVMANGTRLEYTDIKSDKTGKAKYVLKDFTLEGTLAADGKTTLKVTEGTVTLSMNISKSGEITVALDDTDSSGNKKSGTWDSDTSTLTISKNSQKTKQLVFTKENTITVQNYNRAGNALEGSPAEIKDLAELKAALK

SEQ ID NO: 7 - DNA, 784 bp, Artificial Sequence
  Synthetic nucleotide
catatggcacagaaaggtgctgagtctattggttccgtttctgtagatctgcccggtgaaatgaaggttctggtgagcaaagaaaaagacaagaacggcaagtacgatctcatcgcaaccgtcgacaagctggagctgaaaggtacttctgataaaaacaacggctctggtgtgctggagggcgtcaaaactaacaagagcaaagtaaagcttacgatctctgacgatctcggtcagaccacgctggaagttttcaaagaggatggcaagaccctcgtgtccaaaaaagtaacttccaaagacaagtcctctacggaagaaaaattcaacgaaaaaggtgaggtgtctgaaaagatcatcaccatggcagacggcacccgtcttgaatacaccggtattaaaagcgatggtaccggtaaagcgaaatatgttctgaaaaacttcactctggaaggcaaagtggctaatgataaaaccaccttggaagtcaaggaaggcaccgttactctgagcatgaatatctccaaatctggtgaagtttccgttgaactgaacgacactgacagcagcgctgcgactaaaaaaactgcagcgtggaattccaaaacttctactttaaccattagcgttaacagcaaaaaaactacccagctggtgttcactaaacaagacacgatcactgtgcagaaatacgactccaacggcaccaacttagaaggcacggcagtcgaaattaaaacccttgatgaactgaaaaacgcgctgaaataagctgagcggatcc

SEQ ID NO: 8 - protein, 255 aa, Artificial Sequence
  Synthetic peptide
MAQKGAESIGSVSVDLPGEMKVLVSKEKDKNGKYDLIATVDKLELKGTSDKNNGSGVLEGVKTNKSKVKLTISDDLGQTTLEVFKEDGKTLVSKKVTSKDKSSTEEKFNEKGEVSEKIITMADGTRLEYTGIKSDGTGKAKYVLKNFTLEGKVANDKTTLEVKEGTVTLSMNISKSGEVSVELNDTDSSAATKKTAAWNSKTSTLTISVNSKKTTQLVFTKQDTITVQKYDSAGTNLEGTAVEIKTLDELKNALK

SEQ ID NO: 9 - DNA, 787 bp, Artificial Sequence
  Synthetic nucleotide
catatggcacagaaaggtgctgagtctattggttccgtttctgtagatctgcccggtggcatgaccgttctggtcagcaaagaaaaagacaaaaacggtaaatacagcctcgaggcgaccgtcgacaagcttgagctgaaaggcacctctgataaaaacaacggttccggcaccctggaaggtgaaaaaactaacaaaagcaaagtgaaactgaccattgctgatgacctcagccagaccaaattcgaaattttcaaagaagatgccaaaaccttagtatccaaaaaagtgaccctgaaagacaagtcctctaccgaagaaaaattcaacgaaaagggtgaaacctctgaaaaaaccatcgtaatggcaaatggtacccgtctggaatacaccgacatcaaaagcgatggctccggcaaagccaaatacgttctgaaagacttcaccctggaaggcaccctcgctgccgacggcaaaaccaccttgaaagttaccgaaggcactgttgttttaagcatgaacatcttaaaatccggtgaaatcaccgttgcgctggatgactctgacaccactcaggccactaaaaaaaccggcaaatgggattctaacacttccactctgaccatcagcgtgaattccaaaaaaactaaaaacatcgtgttcaccaaagaagacaccatcaccgtccagaaatacgactctgcgggcaccaacctcgaaggcaacgcagtcgaaatcaaaaccctggatgaactgaaaaacgctctgaaataagctgagcggatcc

SEQ ID NO: 10 - protein, 256 aa, Artificial Sequence
  Synthetic peptide
MAQKGAESIGSVSVDLPGGMTVLVSKEKDKNGKYSLEATVDKLELKGTSDKNNGSGTLEGEKTNKSKVKLTIADDLSQTKFEIFKEDAKTLVSKKVTLKDKSSTEEKFNEKGETSEKTIVMANGTRLEYTDIKSDGSGKAKYVLKDFTLEGTLAADGKTTLKVTEGTVVLSMNILKSGEITVALDDSDTTQATKKTGKWDSNTSTLTISVNSKKTKNIVFTKEDTITVQKYDSAGTNLEGNAVEIKTLDELKNALK

SEQ ID NO: 11 - DNA, 784 bp, Artificial Sequence
  Synthetic nucleotide
catatggcacagaaaggtgctgagtctattggttccgtttctgtagatctgcccgggggtatgaaagttctggtaagcaaagaaaaagacaaaaacggtaaatacagcctgatggcaaccgtagaaaagctggagcttaaaggcacttctgataaaaacaacggttctggcaccctggaaggtgaaaaaactaacaaaagcaaagtaaagcttactattgctgaggatctgagcaaaaccacctttgaaatcttcaaagaagatggcaaaactctggtatctaaaaaagtaaccctgaaagacaagtcttctaccgaagaaaaattcaacgaaaagggtgaaatctctgaaaaaactatcgtaatggcaaatggtacccgtctggaatacaccgacatcaaaagcgataaaaccggcaaagctaaatacgttctgaaagactttactctggaaggcactctggctgctgacggcaaaaccactctgaaagttaccgaaggcactgttactctgagcatgaacatttctaaatccggcgaaatcaccgttgcactggatgacactgactctagcggcaataaaaaatccggcacctgggattctgatacttctactttaaccattagcaaaaacagccagaaaactaaacagctggtattcaccaaagaaaacactatcaccgtacagaactataaccgtgcaggcaatgcgctggaaggcagcccggctgaaattaaagatctggcagagctgaaagccgctttgaaataagctgagcggatcc

SEQ ID NO: 12 - protein, 255 aa, Artificial Sequence
  Synthetic peptide
MAQKGAESIGSVSVDLPGGMKVLVSKEKDKNGKYSLMATVEKLELKGTSDKNNGSGTLEGEKTNKSKVKLTIAEDLSKTTFEIFKEDGKTLVSKKVTLKDKSSTEEKFNEKGEISEKTIVMANGTRLEYTDIKSDKTGKAKYVLKDFTLEGTLAADGKTTLKVTEGTVTLSMNISKSGEITVALDDTDSSGNKKSGTWDSDTSTLTISKNSQKTKQLVFTKENTITVQNYNRAGNALEGSPAEIKDLAELKAALK

SEQ ID NO: 13 - protein, 15 aa, Artificial Sequence
  Synthetic peptide
MRLLIGFALALALIG

SEQ ID NO: 14 - DNA, 20 bp, Artificial Sequence
  Synthetic nucleotide
tcggggctggcttaactatg

SEQ ID NO: 15 - DNA, 15 bp, Artificial Sequence
  Synthetic nucleotide
gcttccggctcgtat

SEQ ID NO: 16 - DNA, 20 bp, Artificial Sequence
  Synthetic nucleotide
gcttccggctcgtatgttgt

SEQ ID NO: 17 - DNA, 22 bp, Artificial Sequence
  Synthetic nucleotide
ttatgctagttattgctcagcg

SEQ ID NO: 18 - DNA, 23 bp, Artificial Sequence
  Synthetic nucleotide
ttcccctctagaaataattttgt

SEQ ID NO: 19 - DNA, 29 bp, Artificial Sequence
  Synthetic nucleotide
ggaattccatatgcgtctgttgatcggct

SEQ ID NO: 20 - DNA, 18 bp, Artificial Sequence
  Synthetic nucleotide
ttggtgcctgcggagtcg

SEQ ID NO: 21 - DNA, 20 bp, Artificial Sequence
  Synthetic nucleotide
aatacgactccgcaggcacc

SEQ ID NO: 22 - DNA, 24 bp, Artificial Sequence
  Synthetic nucleotide
ctgggatccgctcagcttatttca

SEQ ID NO: 23 - DNA, 36 bp, Artificial Sequence
  Synthetic nucleotide
cgtgcgtaccatatggcacagaaaggtgctgagtct

SEQ ID NO: 24 - protein, 9 aa, Artificial Sequence
  Synthetic peptide
YVLEGTLTA

SEQ ID NO: 25 - protein, 6 aa, Artificial Sequence
  Synthetic peptide
KEKDKN

SEQ ID NO: 26 - protein, 6 aa, Artificial Sequence
  Synthetic peptide
KTNKSK

SEQ ID NO: 27 - protein, 6 aa, Artificial Sequence
  Synthetic peptide
KEKNKD

SEQ ID NO: 28 - protein, 6 aa, Artificial Sequence
  Synthetic peptide
KEKDKD

SEQ ID NO: 29 - protein, 6 aa, Artificial Sequence
  Synthetic peptide
KADKSK

SEQ ID NO: 30 - protein, 6 aa, Artificial Sequence
  Synthetic peptide
KTDKSK

SEQ ID NO: 31 - DNA, 60 bp, Artificial Sequence
  Synthetic nucleotide
catatgcgtctgttgatcggctttgctctggcgctggctctgatcggctgcgcacagaaa

SEQ ID NO: 32 - DNA, 15 bp, Artificial Sequence
  Synthetic nucleotide
catatggcacagaaa

SEQ ID NO: 33 - protein, 19 aa, Artificial Sequence
  Synthetic peptide
MRLLIGFALALALIGCAQK

SEQ ID NO: 34 - protein, 4 aa, Artificial Sequence
  Synthetic peptide
MAQK

SEQ ID NO: 35 - DNA, 50 bp, Artificial Sequence
  Synthetic nucleotide
gcaaaaacagccagaaaactaaacagctggtattcaccaaagaaaacact

SEQ ID NO: 36 - DNA, 31 bp, Artificial Sequence
  Synthetic nucleotide
gcaaaaacagccagaaaactaaacagctggg

SEQ ID NO: 37 - DNA, 35 bp, Artificial Sequence
  Synthetic nucleotide
aattcaaacagctggtattcaccaaagaaaacact

SEQ ID NO: 38 - DNA, 55 bp, Artificial Sequence
  Synthetic nucleotide
gatcactgtgcagaaatacgactccaacggcaccaacttagaaggcacggcagtc

SEQ ID NO: 39 - DNA, 55 bp, Artificial Sequence
  Synthetic nucleotide
gatcactgtgcagaaatacgactccgcaggcaccaacttagaaggcacggcagtc

SEQ ID NO: 40 - DNA, 52 bp, Artificial Sequence
  Synthetic nucleotide
gatcactgtgcagaaatacgactccggcaccaacttagaaggcacggcagtc

SEQ ID NO: 41 - DNA, 18 bp, Artificial Sequence
  Synthetic nucleotide
cgactccgcaggcaccaa

SEQ ID NO: 42 - DNA, 813 bp, Artificial Sequence
  Synthetic nucleotide
atgagattattaataggatttgctttagcgttagctttaataggatgtgcacaaaaaggtgctgagtcaattggatccgtttcagtagatttgcctggtgaaatgaaagttcttgtaagcaaagaaaaagacaaaaacggcaagtacgatctaattgcaacagtagacaagcttgagcttaaaggaacttctgataaaaacaatggatctggagtacttgaaggcgtaaaaactaacaaaagtaaagtaaaattaacaatttctgacgatctaggtcaaaccacacttgaagttttcaaagaagatggcaaaacactagtatcaaaaaaagtaacttccaaagacaagtcatcaacagaagaaaaattcaatgaaaaaggtgaagtatctgaaaaaataataacaatggcagacggaaccagacttgaatacacaggaattaaaagcgatggaactggaaaagctaaatatgttttaaaaaattttactcttgaaggaaaagtagctaatgataaaacaacattggaagtaaaagaaggaaccgttactttaagtatgaatatttcaaaatctggggaagtttcagttgaacttaatgacactgacagtagtgctgctactaaaaaaactgcagcttggaattcaaaaacttctactttaacaattagtgttaacagcaaaaaaactacacaacttgtgtttactaaacaagacacaataactgtacaaaaatacgactccaacggtaccaatttagaaggcacagcagtcgaaattaaaacacttgatgaacttaaaaacgctttaaaataa

SEQ ID NO: 43 - DNA, 826 bp, Artificial Sequence
  Synthetic nucleotide
atgcgtctgttgatcggctttgctctggcgctggctctgatcggctgcgcacagaaaggtgctgagtctattggttccgtttctgtagatctgcccggtgaaatgaaggttctggtgagcaaagaaaaagacaagaacggcaagtacgatctcatcgcaaccgtcgacaagctggagctgaaaggtacttctgataaaaacaacggctctggtgtgctggagggcgtcaaaactaacaagagcaaagtaaagcttacgatctctgacgatctcggtcagaccacgctggaagttttcaaagaggatggcaagaccctcgtgtccaaaaaagtaacttccaaagacaagtcctctacggaagaaaaattcaacgaaaaaggtgaggtgtctgaaaagatcatcaccatggcagacggcacccgtcttgaatacaccggtattaaaagcgatggtaccggtaaagcgaaatatgttctgaaaaacttcactctggaaggcaaagtggctaatgataaaaccaccttggaagtcaaggaaggcaccgttactctgagcatgaatatctccaaatctggtgaagtttccgttgaactgaacgacactgacagcagcgctgcgactaaaaaaactgcagcgtggaattccaaaacttctactttaaccattagcgttaacagcaaaaaaactacccagctggtgttcactaaacaagacacgatcactgtgcagaaatacgactccgcaggcaccaacttagaaggcacggcagtcgaaattaaaacccttgatgaactgaaaaacgcgctgaaataagctgagcggatcc

SEQ ID NO: 44 - DNA, 818 bp, Artificial Sequence
  Synthetic nucleotide
atatgagattattaataggatttgctttagcgttagctttaataggatgtgcacaaaaaggtgctgagtcaattggatccgtttcagtagatttacctggtggaatgacagttcttgtaagtaaagaaaaagacaaagacggtaaatacagtctagaggcaacagtagacaagcttgagcttaaaggaacttctgataaaaacaacggttctggaacacttgaaggtgaaaaaactgacaaaagtaaagtaaaattaacaattgctgatgacctaagtcaaactaaatttgaaattttcaaagaagatgccaaaacattagtatcaaaaaaagtaacccttaaagacaagtcatcaacagaagaaaaattcaacgaaaagggtgaaacatctgaaaaaacaatagtaagagcaaatggaaccagacttgaatacacagacataaaaagcgatggatccggaaaagctaaagaagttttaaaagactttactcttgaaggaactctagctgctgacggcaaaacaacattgaaagttacagaaggcactgttgttttaagcaagaacattttaaaatccggagaaataacagttgcacttgatgactctgacactactcaggctactaaaaaaactggaaaatgggattcaaatacttccactttaacaattagtgtgaatagcaaaaaaactaaaaacattgtatttacaaaagaagacacaataacagtacaaaaatacgactcagcaggcaccaatctagaaggcaacgcagtcgaaattaaaacacttgatgaacttaaaaacgctttaaaataa

SEQ ID NO: 45 - DNA, 831 bp, Artificial Sequence
  Synthetic nucleotide
atatgcgtctgttgatcggctttgctctggcgctggctctgatcggctgcgcacagaaaggtgctgagtctattggttccgtttctgtagatctgcccggtggcatgaccgttctggtcagcaaagaaaaagacaaaaacggtaaatacagcctcgaggcgaccgtcgacaagcttgagctgaaaggcacctctgataaaaacaacggttccggcaccctggaaggtgaaaaaactaacaaaagcaaagtgaaactgaccattgctgatgacctcagccagaccaaattcgaaattttcaaagaagatgccaaaaccttagtatccaaaaaagtgaccctgaaagacaagtcctctaccgaagaaaaattcaacgaaaagggtgaaacctctgaaaaaaccatcgtaatggcaaatggtacccgtctggaatacaccgacatcaaaagcgatggctccggcaaagccaaatacgttctgaaagacttcaccctggaaggcaccctcgctgccgacggcaaaaccaccttgaaagttaccgaaggcactgttgttttaagcatgaacatcttaaaatccggtgaaatcaccgttgcgctggatgactctgacaccactcaggccactaaaaaaaccggcaaatgggattctaacacttccactctgaccatcagcgtgaattccaaaaaaactaaaaacatcgtgttcaccaaagaagacaccatcaccgtccagaaatacgactctgcgggcaccaacctcgaaggcaacgcagtcgaaatcaaaaccctggatgaactgaaaaacgctctgaaataagctgagcggatcc

SEQ ID NO: 46 - DNA, 816 bp, Artificial Sequence
  Synthetic nucleotide
catatgagattattaataggatttgctttagcgttagctttaataggatgtgcacaaaaaggtgctgagtcaattggatccgtttcagtagatttacctggtggaatgaaagttcttgtaagtaaagaaaaagacaaagatggtaaatacagtctaatggcaacagtagaaaagcttgagcttaaaggaacttctgataaaaacaacggttctggaacacttgaaggtgaaaaaactgacaaaagtaaagtaaaattaacaattgctgaggatctaagtaaaaccacatttgaaatcttcaaagaagatggcaaaacattagtatcaaaaaaagtaacccttaaagacaagtcatcaacagaagaaaaattcaacgaaaagggtgaaatatctgaaaaaacaatagtaagagcaaatggaaccagacttgaatacacagacataaaaagcgataaaaccggaaaagctaaagaagttttaaaagactttactcttgaaggaactctagctgctgacggcaaaacaacattgaaagttacagaaggcactgttactttaagcaagaacatttcaaaatccggagaaataacagttgcacttgatgacactgactctagcggcaataaaaaatccggaacatgggattcagatacttctactttaacaattagtaaaaacagtcaaaaaactaaacaacttgtattcacaaaagaaaacacaataacagtacaaaactataacagagcaggcaatgcgcttgaaggcagcccagctgaaattaaagatcttgcagagcttaaagccgctttaaaataa

SEQ ID NO: 47 - DNA, 829 bp, Artificial Sequence; identical to SEQ ID NO: 5
  Synthetic peptide

SEQ ID NO: 48 - DNA, 829 bp, Artificial Sequence
  Synthetic nucleotide
ggatccgctcagcttatttcagcgcgtttttcagttcatcaagggttttaatttcgactgccgtgccttctaagttggtgcctgcggagtcgtatttctgcacagtgatcgtgtcttgtttagtgaacaccagctgggtagtttttttgctgttaacgctaatggttaaagtagaagttttggaattccacgctgcagtttttttagtcgcagcgctgctgtcagtgtcgttcagttcaacggaaacttcaccagatttggagatattcatgctcagagtaacggtgccttccttgacttccaaggtggttttatcattagccactttgccttccagagtgaagtttttcagaacatatttcgctttaccggtaccatcgcttttaataccggtgtattcaagacgggtgccgtctgccatggtgatgatcttttcagacacctcacctttttcgttgaatttttcttccgtagaggacttgtctttggaagttacttttttggacacgagggtcttgccatcctctttgaaaacttccagcgtggtctgaccgagatcgtcagagatcgtaagctttactttgctcttgttagttttgacgccctccagcacaccagagccgttgtttttatcagaagtacctttcagctccagcttgtcgacggttgcgatgagatcgtacttgccgttcttgtctttttctttgctcaccagaaccttcatttcaccgggcagatctacagaaacggaaccaatagactcagcacctttctgtgcgcagccgatcagagccagcgccagagcaaagccgatcaacagacgcatatg

SEQ ID NO: 49 - DNA, 832 bp, Artificial Sequence
  Synthetic nucleotide
ggatccgctcagcttatttcagagcgtttttcagttcatccagggttttgatttcgactgcgttgccttcgaggttggtgcccgcagagtcgtatttctggacggtgatggtgtcttctttggtgaacacgatgtttttagtttttttggaattcacgctgatggtcagagtggaagtgttagaatcccatttgccggtttttttagtggcctgagtggtgtcagagtcatccagcgcaacggtgatttcaccggattttaagatgttcatgcttaaaacaacagtgccttcggtaactttcaaggtggttttgccgtcggcagcgagggtgccttccagggtgaagtctttcagaacgtatttggctttgccggagccatcgcttttgatgtcggtgtattccagacgggtaccatttgccattacgatggttttttcagaggtttcacccttttcgttgaatttttcttcggtagaggacttgtctttcagggtcacttttttggatactaaggttttggcatcttctttgaaaatttcgaatttggtctggctgaggtcatcagcaatggtcagtttcactttgcttttgttagttttttcaccttccagggtgccggaaccgttgtttttatcagaggtgcctttcagctcaagcttgtcgacggtcgcctcgaggctgtatttaccgtttttgtctttttctttgctgaccagaacggtcatgccaccgggcagatctacagaaacggaaccaatagactcagcacctttctgtgcgcagccgatcagagccagcgccagagcaaagccgatcaacagacgcatatg

SEQ ID NO: 50 - DNA, 829 bp, Artificial Sequence
  Synthetic nucleotide
ggatccgctcagcttatttcaaagcggctttcagctctgccagatctttaatttcagccgggctgccttccagcgcattgcctgcacggttatagttctgtacggtgatagtgttttctttggtgaataccagctgtttagttttctggctgtttttgctaatggttaaagtagaagtatcagaatcccaggtgccggattttttattgccgctagagtcagtgtcatccagtgcaacggtgatttcgccggatttagaaatgttcatgctcagagtaacagtgccttcggtaactttcagagtggttttgccgtcagcagccagagtgccttccagagtaaagtctttcagaacgtatttagctttgccggttttatcgcttttgatgtcggtgtattccagacgggtaccatttgccattacgatagttttttcagagatttcacccttttcgttgaatttttcttcggtagaagacttgtctttcagggttacttttttagataccagagttttgccatcttctttgaagatttcaaaggtggttttgctcagatcctcagcaatagtaagctttactttgcttttgttagttttttcaccttccagggtgccagaaccgttgtttttatcagaagtgcctttaagctccagcttttctacggttgccatcaggctgtatttaccgtttttgtctttttctttgcttaccagaactttcatacccccgggcagatctacagaaacggaaccaatagactcagcacctttctgtgcacagccgattaaagccagcgccaaagcaaagccgatcaacagacgcatatg

SEQ ID NO: 51 - DNA, 60 bp, Artificial Sequence
  Synthetic nucleotide
tttctgtgcgcagccgatcagagccagcgccagagcaaagccgatcaacagacgcatatg

SEQ ID NO: 52 - DNA, 15 bp, Artificial Sequence
  Synthetic nucleotide
tttctgtgccatatg

SEQ ID NO: 53 - DNA, 50 bp, Artificial Sequence
  Synthetic nucleotide
agtgttttctttggtgaataccagctgtttagttttctggctgtttttgc

SEQ ID NO: 54 - DNA, 35 bp, Artificial Sequence
  Synthetic nucleotide
aattcccagctgtttagttttctggctgtttttgc

SEQ ID NO: 55 - DNA, 784 bp, Artificial Sequence
  Synthetic nucleotide
gtataccgtgtctttccacgactcagataaccaaggcaaagacatctagacgggccactttacttccaagaccactcgtttctttttctgttcttgccgttcatgctagagtagcgttggcagctgttcgacctcgactttccatgaagactatttttgttgccgagaccacacgacctcccgcagttttgattgttctcgtttcatttcgaatgctagagactgctagagccagtctggtgcgaccttcaaaagtttctcctaccgttctgggagcacaggttttttcattgaaggtttctgttcaggagatgccttctttttaagttgctttttccactccacagacttttctagtagtggtaccgtctgccgtgggcagaacttatgtggccataattttcgctaccatggccatttcgctttatacaagactttttgaagtgagaccttccgtttcaccgattactattttggtggaaccttcagttccttccgtggcaatgagactcgtacttatagaggtttagaccacttcaaaggcaacttgacttgctgtgactgtcgtcgcgacgctgatttttttgacgtcgcaccttaaggttttgaagatgaaattggtaatcgcaattgtcgtttttttgatgggtcgaccacaagtgatttgttctgtgctagtgacacgtctttatgctgaggttgccgtggttgaatcttccgtgccgtcagctttaattttgggaactacttgactttttgcgcgactttattcgactcgcctagg

SEQ ID NO: 56 - DNA, 787 bp, Artificial Sequence
  Sythetic nucleotide
gtataccgtgtctttccacgactcagataaccaaggcaaagacatctagacgggccaccgtactggcaagaccagtcgtttctttttctgtttttgccatttatgtcggagctccgctggcagctgttcgaactcgactttccgtggagactatttttgttgccaaggccgtgggaccttccacttttttgattgttttcgtttcactttgactggtaacgactactggagtcggtctggtttaagctttaaaagtttcttctacggttttggaatcataggttttttcactgggactttctgttcaggagatggcttctttttaagttgcttttcccactttggagacttttttggtagcattaccgtttaccatgggcagaccttatgtggctgtagttttcgctaccgaggccgtttcggtttatgcaagactttctgaagtgggaccttccgtgggagcgacggctgccgttttggtggaactttcaatggcttccgtgacaacaaaattcgtacttgtagaattttaggccactttagtggcaacgcgacctactgagactgtggtgagtccggtgatttttttggccgtttaccctaagattgtgaaggtgagactggtagtcgcacttaaggtttttttgatttttgtagcacaagtggtttcttctgtggtagtggcaggtctttatgctgagacgcccgtggttggagcttccgttgcgtcagctttagttttgggacctacttgactttttgcgagactttattcgactcgcctagg

SEQ ID NO: 57 - DNA, 784 bp, Artificial Sequence
  Synthetic nucleotide
gtataccgtgtctttccacgactcagataaccaaggcaaagacatctagacgggcccccatactttcaagaccattcgtttctttttctgtttttgccatttatgtcggactaccgttggcatcttttcgacctcgaatttccgtgaagactatttttgttgccaagaccgtgggaccttccacttttttgattgttttcgtttcatttcgaatgataacgactcctagactcgttttggtggaaactttagaagtttcttctaccgttttgagaccatagattttttcattgggactttctgttcagaagatggcttctttttaagttgcttttcccactttagagacttttttgatagcattaccgtttaccatgggcagaccttatgtggctgtagttttcgctattttggccgtttcgatttatgcaagactttctgaaatgagaccttccgtgagaccgacgactgccgttttggtgagactttcaatggcttccgtgacaatgagactcgtacttgtaaagatttaggccgctttagtggcaacgtgacctactgtgactgagatcgccgttattttttaggccgtggaccctaagactatgaagatgaaattggtaatcgtttttgtcggtcttttgatttgtcgaccataagtggtttcttttgtgatagtggcatgtcttgatattggcacgtccgttacgcgaccttccgtcgggccgactttaatttctagaccgtctcgactttcggcgaaactttattcgactcgcctagg

SEQ ID NO: 58 - DNA, 31 bp, Artificial Sequence
  Synthetic nucleotide
agtgttttctttggtgaataccagctgtttg

SEQ ID NO: 59 - DNA, 45 bp, Artificial Sequence
  Synthetic nucleotide
tatgcgtctgttgatcggctttgctctggcgctggctctgatcgg

SEQ ID NO: 60 - DNA, 50 bp, Artificial Sequence
  Synthetic nucleotide
ctgcgcacagaaaggtgctgagtctattggttccgtttctgtagatctgc

SEQ ID NO: 61 - DNA, 50 bp, Artificial Sequence
  Synthetic nucleotide
ccggtgaaatgaaggttctggtgagcaaagaaaaagacaagaacggcaag

SEQ ID NO: 62 - DNA, 50 bp, Artificial Sequence
  Synthetic nucleotide
tacgatctcatcgcaaccgtcgacaagctggagctgaaaggtacttctga

SEQ ID NO: 63 - DNA, 56 bp, Artificial Sequence
  Synthetic nucleotide
taaaaacaacggctctggtgtgctggagggcgtcaaaactaacaagagcaaagtaa

SEQ ID NO: 64 - DNA, 40 bp, Artificial Sequence
  Synthetic nucleotide
agctttactttgctcttgttagttttgacgccctccagca

SEQ ID NO: 65 - DNA, 50 bp, Artificial Sequence
  Synthetic nucleotide
caccagagccgttgtttttatcagaagtacctttcagctccagcttgtcg

SEQ ID NO: 66 - DNA, 50 bp, Artificial Sequence
  Synthetic nucleotide
acggttgcgatgagatcgtacttgccgttcttgtctttttctttgctcac

SEQ ID NO: 67 - DNA, 50 bp, Artificial Sequence
  Synthetic nucleotide
cagaaccttcatttcaccgggcagatctacagaaacggaaccaatagact

SEQ ID NO: 68 - DNA, 63 bp, Artificial Sequence
  Synthetic nucleotide
cagcacctttctgtgcgcagccgatcagagccagcgccagagcaaagccgatcaacagacgca

SEQ ID NO: 69 - DNA, 34 bp, Artificial Sequence
  Synthetic nucleotide
agcttacgatctctgacgatctcggtcagaccac

SEQ ID NO: 70 - DNA, 50 bp, Artificial Sequence
  Synthetic nucleotide
gctggaagttttcaaagaggatggcaagaccctcgtgtccaaaaaagtaa

SEQ ID NO: 71 - DNA, 50 bp, Artificial Sequence
  Synthetic nucleotide
cttccaaagacaagtcctctacggaagaaaaattcaacgaaaaaggtgag

SEQ ID NO: 72 - DNA, 40 bp, Artificial Sequence
  Synthetic nucleotide
gtgtctgaaaagatcatcaccatggcagacggcacccgtc

SEQ ID NO: 73 - DNA, 31 bp, Artificial Sequence
  Synthetic nucleotide
ttgaatacaccggtattaaaagcgatggtac

SEQ ID NO: 74 - DNA, 47 bp, Artificial Sequence
  Synthetic nucleotide
catcgcttttaataccggtgtattcaagacgggtgccgtctgccatg

SEQ ID NO: 75 - DNA, 50 bp, Artificial Sequence
  Synthetic nucleotide
gtgatgatcttttcagacacctcacctttttcgttgaatttttcttccgt

SEQ ID NO: 76 - DNA, 50 bp, Artificial Sequence
  Synthetic nucleotide
agaggacttgtctttggaagttacttttttggacacgagggtcttgccat

SEQ ID NO: 77 - DNA, 50 bp, Artificial Sequence
  Synthetic nucleotide
cctctttgaaaacttccagcgtggtctgaccgagatcgtcagagatcgta

SEQ ID NO: 78 - DNA, 39 bp, Artificial Sequence
  Synthetic nucleotide
cggtaaagcgaaatatgttctgaaaaacttcactctgga

SEQ ID NO: 79 - DNA, 50 bp, Artificial Sequence
  Synthetic nucleotide
aggcaaagtggctaatgataaaaccaccttggaagtcaaggaaggcaccg

SEQ ID NO: 80 - DNA, 50 bp, Artificial Sequence
  Synthetic nucleotide
ttactctgagcatgaatatctccaaatctggtgaagtttccgttgaactg

SEQ ID NO: 81 - DNA, 45 bp, Artificial Sequence
  Synthetic nucleotide
aacgacactgacagcagcgctgcgactaaaaaaactgcagcgtgg

SEQ ID NO: 82 - DNA, 29 bp, Artificial Sequence
  Synthetic nucleotide
aattccacgctgcagtttttttagtcgca

SEQ ID NO: 83 - DNA, 50 bp, Artificial Sequence
  Synthetic nucleotide
gcgctgctgtcagtgtcgttcagttcaacggaaacttcaccagatttgga

SEQ ID NO: 84 - DNA, 50 bp, Artificial Sequence
  Synthetic nucleotide
gatattcatgctcagagtaacggtgccttccttgacttccaaggtggttt

SEQ ID NO: 85 - DNA, 63 bp, Artificial Sequence
  Synthetic nucleotide
tatcattagccactttgccttccagagtgaagtttttcagaacatatttcgctttaccggtac

SEQ ID NO: 86 - DNA, 45 bp, Artificial Sequence
  Synthetic nucleotide
aattccaaaacttctactttaaccattagcgttaacagcaaaaaa

SEQ ID NO: 87 - DNA, 50 bp, Artificial Sequence
  Synthetic nucleotide
actacccagctggtgttcactaaacaagacacgatcactgtgcagaaata

SEQ ID NO: 88 - DNA, 50 bp, Artificial Sequence
  Synthetic nucleotide
cgactccaacggcaccaacttagaaggcacggcagtcgaaattaaaaccc

SEQ ID NO: 89 - DNA, 37 bp, Artificial Sequence
  Synthetic nucleotide
ttgatgaactgaaaaacgcgctgaaataagctgagcg

SEQ ID NO: 90 - DNA, 61 bp, Artificial Sequence
  Synthetic nucleotide
gatccgctcagcttatttcagcgcgtttttcagttcatcaagggttttaatttcgactgcc

SEQ ID NO: 91 - DNA, 50 bp, Artificial Sequence
  Synthetic nucleotide
gtgccttctaagttggtgccgttggagtcgtatttctgcacagtgatcgt

SEQ ID NO: 92 - DNA, 50 bp, Artificial Sequence
  Synthetic nucleotide
gtcttgtttagtgaacaccagctgggtagtttttttgctgttaacgctaa

SEQ ID NO: 93 - DNA, 21 bp, Artificial Sequence
  Synthetic nucleotide
tggttaaagtagaagttttgg

SEQ ID NO: 94 - DNA, 48 bp, Artificial Sequence
  Synthetic nucleotide
tatgcgtctgttgatcggctttgctttggcgctggctttaatcggctg

SEQ ID NO: 95 - DNA, 50 bp, Artificial Sequence
  Synthetic nucleotide
tgcacagaaaggtgctgagtctattggttccgtttctgtagatctgcccg

SEQ ID NO: 96 - DNA, 50 bp, Artificial Sequence
  Synthetic nucleotide
ggggtatgaaagttctggtaagcaaagaaaaagacaaaaacggtaaatac

SEQ ID NO: 97 - DNA, 50 bp, Artificial Sequence
  Synthetic nucleotide
agcctgatggcaaccgtagaaaagctggagcttaaaggcacttctgataa

SEQ ID NO: 98 - DNA, 53 bp, Artificial Sequence
  Synthetic nucleotide
aaacaacggttctggcaccctggaaggtgaaaaaactaacaaaagcaaagtaa

SEQ ID NO: 99 - DNA, 37 bp, Artificial Sequence
  Synthetic nucleotide
agctttactttgcttttgttagttttttcaccttcca

SEQ ID NO: 100 - DNA, 50 bp, Artificial Sequence
  Synthetic nucleotide
gggtgccagaaccgttgtttttatcagaagtgcctttaagctccagcttt

SEQ ID NO: 101 - DNA, 50 bp, Artificial Sequence
  Synthetic nucleotide
tctacggttgccatcaggctgtatttaccgtttttgtctttttctttgct

SEQ ID NO: 102 - DNA, 50 bp, Artificial Sequence
  Synthetic nucleotide
taccagaactttcatacccccgggcagatctacagaaacggaaccaatag

SEQ ID NO: 103 - DNA, 30 bp, Artificial Sequence
  Synthetic nucleotide
actcagcacctttctgtgcacagccgatta

SEQ ID NO: 104 - DNA, 36 bp, Artificial Sequence
  Synthetic nucleotide
aagccagcgccaaagcaaagccgatcaacagacgca

SEQ ID NO: 105 - DNA, 47 bp, Artificial Sequence
  Synthetic nucleotide
agcttactattgctgaggatctgagcaaaaccacctttgaaatcttc

SEQ ID NO: 106 - DNA, 50 bp, Artificial Sequence
  Synthetic nucleotide
aaagaagatggcaaaactctggtatctaaaaaagtaaccctgaaagacaa

SEQ ID NO: 107 - DNA, 40 bp, Artificial Sequence
  Synthetic nucleotide
gtcttctaccgaagaaaaattcaacgaaaagggtgaaatc

SEQ ID NO: 108 - DNA, 32 bp, Artificial Sequence
  Synthetic nucleotide
tctgaaaaaactatcgtaatggcaaatggtac

SEQ ID NO: 109 - DNA, 33 bp, Artificial Sequence
  Synthetic nucleotide
aaggtggttttgctcagatcctcagcaatagta

SEQ ID NO: 110 - DNA, 30 bp, Artificial Sequence
  Synthetic nucleotide
agagttttgccatcttctttgaagatttca

SEQ ID NO: 111 - DNA, 50 bp, Artificial Sequence
  Synthetic nucleotide
atttttcttcggtagaagacttgtctttcagggttacttttttagatacc

SEQ ID NO: 112 - DNA, 48 bp, Artificial Sequence
  Synthetic nucleotide
catttgccattacgatagttttttcagagatttcacccttttcgttga

SEQ ID NO: 113 - DNA, 48 bp, Artificial Sequence
  Synthetic nucleotide
ccgtctggaatacaccgacatcaaaagcgataaaaccggcaaagctaa

SEQ ID NO: 114 - DNA, 50 bp, Artificial Sequence
  Synthetic nucleotide
atacgttctgaaagactttactctggaaggcactctggctgctgacggca

SEQ ID NO: 115 - DNA, 50 bp, Artificial Sequence
  Synthetic nucleotide
aaaccactctgaaagttaccgaaggcactgttactctgagcatgaacatt

SEQ ID NO: 116 - DNA, 50 bp, Artificial Sequence
  Synthetic nucleotide
tctaaatccggcgaaatcaccgttgcactggatgacactgactctagcgg

SEQ ID NO: 117 - DNA, 50 bp, Artificial Sequence
  Synthetic nucleotide
caataaaaaatccggcacctgggattctgatacttctactttaaccatta

SEQ ID NO: 118 - DNA, 31 bp, Artificial Sequence; identical to SEQ ID NO: 36
  Synthetic nucleotide

SEQ ID NO: 119 - DNA, 32 bp, Artificial Sequence
  Synthetic nucleotide
gcttttgatgtcggtgtattccagacgggtac

SEQ ID NO: 120 - DNA, 50 bp, Artificial Sequence
  Synthetic nucleotide
ccttccagagtaaagtctttcagaacgtatttagctttgccggttttatc

SEQ ID NO: 121 - DNA, 50 bp, Artificial Sequence
  Synthetic nucleotide
cagtgccttcggtaactttcagagtggttttgccgtcagcagccagagtg

SEQ ID NO: 122 - DNA, 50 bp, Artificial Sequence
  Synthetic nucleotide
cagtgcaacggtgatttcgccggatttagaaatgttcatgctcagagtaa

SEQ ID NO: 123 - DNA, 50 bp, Artificial Sequence
  Synthetic nucleotide
tcagaatcccaggtgccggattttttattgccgctagagtcagtgtcatc

SEQ ID NO: 124 - DNA, 55 bp, Artificial Sequence
  Synthetic nucleotide
aattcccagctgtttagttttctggctgtttttgctaatggttaaagtagaagta

SEQ ID NO: 125 - DNA, 45 bp, Artificial Sequence
  Synthetic nucleotide
aattcaaacagctggtattcaccaaagaaaacactatcaccgtac

SEQ ID NO: 126 - DNA, 40 bp, Artificial Sequence
  Synthetic nucleotide
agaactataaccgtgcaggcaatgcgctggaaggcagccc

SEQ ID NO: 127 - DNA, 54 bp, Artificial Sequence
  Synthetic nucleotide
ggctgaaattaaagatctggcagagctgaaagccgctttgaaataagctgagcg

SEQ ID NO: 128 - DNA, 28 bp, Artificial Sequence
  Synthetic nucleotide
gatccgctcagcttatttcaaagcggct

SEQ ID NO: 129 - DNA, 50 bp, Artificial Sequence
  Synthetic nucleotide
ttcagctctgccagatctttaatttcagccgggctgccttccagcgcatt

SEQ ID NO: 130 - DNA, 61 bp, Artificial Sequence
  Synthetic nucleotide
gcctgcacggttatagttctgtacggtgatagtgttttctttggtgaataccagctgtttg

SEQ ID NO: 131 - DNA, 48 bp, Artificial Sequence
  Synthetic nucleotide
tatgcgtctgttgatcggctttgctctggcgctggctctgatcggctg

SEQ ID NO: 132 - DNA, 50 bp, Artificial Sequence
  Synthetic nucleotide
cgcacagaaaggtgctgagtctattggttccgtttctgtagatctgcccg

SEQ ID NO: 133 - DNA, 42 bp, Artificial Sequence
  Synthetic nucleotide
gtggcatgaccgttctggtcagcaaagaaaaagacaaaaacg

SEQ ID NO: 134 - DNA, 30 bp, Artificial Sequence
  Synthetic nucleotide
gtaaatacagcctcgaggcgaccgtcgaca

SEQ ID NO: 135 - DNA, 56 bp, Artificial Sequence
  Synthetic nucleotide
agcttgtcgacggtcgcctcgaggctgtatttaccgtttttgtctttttctttgct

SEQ ID NO: 136 - DNA, 40 bp, Artificial Sequence
  Synthetic nucleotide
gaccagaacggtcatgccaccgggcagatctacagaaacg

SEQ ID NO: 137 - DNA, 50 bp, Artificial Sequence
  Synthetic nucleotide
gaaccaatagactcagcacctttctgtgcgcagccgatcagagccagcgc

SEQ ID NO: 138 - DNA, 26 bp, Artificial Sequence
  Synthetic nucleotide
cagagcaaagccgatcaacagacgca

SEQ ID NO: 139 - DNA, 50 bp, Artificial Sequence
  Synthetic nucleotide
agcttgagctgaaaggcacctctgataaaaacaacggttccggcaccctg

SEQ ID NO: 140 - DNA, 48 bp, Artificial Sequence
  Synthetic nucleotide
gaaggtgaaaaaactaacaaaagcaaagtgaaactgaccattgctgat

SEQ ID NO: 141 - DNA, 50 bp, Artificial Sequence
  Synthetic nucleotide
gacctcagccagaccaaattcgaaattttcaaagaagatgccaaaacctt

SEQ ID NO: 142 - DNA, 50 bp, Artificial Sequence
  Synthetic nucleotide
agtatccaaaaaagtgaccctgaaagacaagtcctctaccgaagaaaaat

SEQ ID NO: 143 - DNA, 52 bp, Artificial Sequence
  Synthetic nucleotide
tcaacgaaaagggtgaaacctctgaaaaaaccatcgtaatggcaaatggtac

SEQ ID NO: 144 - DNA, 28 bp, Artificial Sequence
  Synthetic nucleotide
catttgccattacgatggttttttcaga

SEQ ID NO: 145 - DNA, 40 bp, Artificial Sequence
  Synthetic nucleotide
ggtttcacccttttcgttgaatttttcttcggtagaggac

SEQ ID NO: 146 - DNA, 50 bp, Artificial Sequence
  Synthetic nucleotide
ttgtctttcagggtcacttttttggatactaaggttttggcatcttcttt

SEQ ID NO: 147 - DNA, 50 bp, Artificial Sequence
  Synthetic nucleotide
gaaaatttcgaatttggtctggctgaggtcatcagcaatggtcagtttca

SEQ ID NO: 148 - DNA, 40 bp, Artificial Sequence
  Synthetic nucleotide
ctttgcttttgttagttttttcaccttccagggtgccgga

SEQ ID NO: 149 - DNA, 34 bp, Artificial Sequence
  Synthetic nucleotide
accgttgtttttatcagaggtgcctttcagctca

SEQ ID NO: 150 - DNA, 48 bp, Artificial Sequence
  Synthetic nucleotide
ccgtctggaatacaccgacatcaaaagcgatggctccggcaaagccaa

SEQ ID NO: 151 - DNA, 48 bp, Artificial Sequence
  Synthetic nucleotide
atacgttctgaaagacttcaccctggaaggcaccctcgctgccgacgg

SEQ ID NO: 152 - DNA, 42 bp, Artificial Sequence
  Synthetic nucleotide
caaaaccaccttgaaagttaccgaaggcactgttgttttaag

SEQ ID NO: 153 - DNA, 40 bp, Artificial Sequence
  Synthetic nucleotide
catgaacatcttaaaatccggtgaaatcaccgttgcgctg

SEQ ID NO: 154 - DNA, 50 bp, Artificial Sequence
  Synthetic nucleotide
gatgactctgacaccactcaggccactaaaaaaaccggcaaatgggattc

SEQ ID NO: 155 - DNA, 28 bp, Artificial Sequence
  Synthetic nucleotide
taacacttccactctgaccatcagcgtg

SEQ ID NO: 156 - DNA, 47 bp, Artificial Sequence
  Synthetic nucleotide
aattcacgctgatggtcagagtggaagtgttagaatcccatttgccg

SEQ ID NO: 157 - DNA, 55 bp, Artificial Sequence
  Synthetic nucleotide
gtttttttagtggcctgagtggtgtcagagtcatccagcgcaacggtgatttcac

SEQ ID NO: 158 - DNA, 50 bp, Artificial Sequence
  Synthetic nucleotide
cggattttaagatgttcatgcttaaaacaacagtgccttcggtaactttc

SEQ ID NO: 159 - DNA, 40 bp, Artificial Sequence
  Synthetic nucleotide
aaggtggttttgccgtcggcagcgagggtgccttccaggg

SEQ ID NO: 160 - DNA, 40 bp, Artificial Sequence
  Synthetic nucleotide
tgaagtctttcagaacgtatttggctttgccggagccatc

SEQ ID NO: 161 - DNA, 32 bp, Artificial Sequence; identical to SEQ ID NO: 119
  Synthetic nucleotide

SEQ ID NO: 162 - DNA, 52 bp, Artificial Sequence
  Synthetic nucleotide
aattccaaaaaaactaaaaacatcgtgttcaccaaagaagacaccatcaccg

SEQ ID NO: 163 - DNA, 50 bp, Artificial Sequence
  Synthetic nucleotide
tccagaaatacgactctgcgggcaccaacctcgaaggcaacgcagtcgaa

SEQ ID NO: 164 - DNA, 47 bp, Artificial Sequence
  Synthetic nucleotide
atcaaaaccctggatgaactgaaaaacgctctgaaataagctgagcg

SEQ ID NO: 165 - DNA, 71 bp, Artificial Sequence
  Synthetic nucleotide
gatccgctcagcttatttcagagcgtttttcagttcatccagggttttgatttcgactgcgttgccttcga

SEQ ID NO: 166 - DNA, 50 bp, Artificial Sequence
  Synthetic nucleotide
ggttggtgcccgcagagtcgtatttctggacggtgatggtgtcttctttg

SEQ ID NO: 167 - DNA, 28 bp, Artificial Sequence
  Synthetic nucleotide
gtgaacacgatgtttttagtttttttgg

SEQ ID NO: 168 - DNA, 822 bp, Artificial Sequence
  Synthetic nucleotide
atgaaaaaatatttattgggaataggtctaatattagccttaatagcatgtaagcaaaatgttagcagccttgacgagaaaaacagcgtttcagtagatttgcctggtgaaatgaaagttcttgtaagcaaagaaaaaaacaaagacggcaagtacgatctaattgcaacagtagacaagcttgagcttaaaggaacttctgataaaaacaatggatctggagtacttgaaggcgtaaaagctgacaaaagtaaagtaaaattaacaatttctgacgatctaggtcaaaccacacttgaagttttcaaagaagatggcaaaacactagtatcaaaaaaagtaacttccaaagacaagtcatcaacagaagaaaaattcaatgaaaaaggtgaagtatctgaaaaaataataacaagagcagacggaaccagacttgaatacacaggaattaaaagcgatggatctggaaaagctaaagaggttttaaaaaactttactcttgaaggaaaagtagctaatgataaagtaacattggaagtaaaagaaggaaccgttactttaagtaaaaatatttcaaaatctggggaagtttcagttgaacttaatgacactgacagtagtgctgctactaaaaaaactgcagcttggaattcaaaaacttctactttaacaattagtgttaacagcaaaaaaactacacaacttgtgtttactaaacaagacacaataactgtacaaaaatacgactccgcaggtaccaatttagaaggcacagcagtcgaaattaaaacacttgatgaacttaaaaacgctttaaaatag

SEQ ID NO: 169 - protein, 273 aa, Artificial Sequence
  Synthetic peptide
MKKYLLGIGLILALIACKQNVSSLDEKNSVSVDLPGEMKVLVSKEKNKDGKYDLIATVDKLELKGTSDKNNGSGVLEGVKADKSKVKLTISDDLGQTTLEVFKEDGKTLVSKKVTSKDKSSTEEKFNEKGEVSEKIITRADGTRLEYTGIKSDGSGKAKEVLKNFTLEGKVANDKVTLEVKEGTVTLSKNISKSGEVSVELNDTDSSAATKKTAAWNSKTSTLTISVNSKKTTQLVFTKQDTITVQKYDSAGTNLEGTAVEIKTLDELKNALK

SEQ ID NO: 170 - DNA, 825 bp, Artificial Sequence
  Synthetic nucleotide
atgaaaaaatatttattgggaataggtctaatattagccttaatagcatgtaagcaaaatgttagcacgcttgatgaaaaaaatagcgtttcagtagatttacctggtggaatgacagttcttgtaagtaaagaaaaagacaaagacggtaaatacagtctagaggcaacagtagacaagcttgagcttaaaggaacttctgataaaaacaacggttctggaacacttgaaggtgaaaaaactgacaaaagtaaagtaaaattaacaattgctgatgacctaagtcaaactaaatttgaaattttcaaagaagatgccaaaacattagtatcaaaaaaagtaacccttaaagacaagtcatcaacagaagaaaaattcaacgaaaagggtgaaacatctgaaaaaacaatagtaagagcaaatggaaccagacttgaatacacagacataaaaagcgatggatccggaaaagctaaagaagttttaaaagactttactcttgaaggaactctagctgctgacggcaaaacaacattgaaagttacagaaggcactgttgttttaagcaagaacattttaaaatccggagaaataacagttgcacttgatgactctgacactactcaggctactaaaaaaactggaaaatgggattcaaatacttccactttaacaattagtgtgaatagcaaaaaaactaaaaacattgtatttacaaaagaagacacaataacagtacaaaaatacgactcagcaggcaccaatctagaaggcaacgcagtcgaaattaaaacacttgatgaacttaaaaacgctttaaaataa

SEQ ID NO: 171 - protein, 274 aa, Artificial Sequence
  Synthetic peptide
MKKYLLGIGLILALIACKQNVSTLDEKNSVSVDLPGGMTVLVSKEKDKDGKYSLEATVDKLELKGTSDKNNGSGTLEGEKTDKSKVKLTIADDLSQTKFEIFKEDAKTLVSKKVTLKDKSSTEEKFNEKGETSEKTIVRANGTRLEYTDIKSDGSGKAKEVLKDFTLEGTLAADGKTTLKVTEGTVVLSKNILKSGEITVALDDSDTTQATKKTGKWDSNTSTLTISVNSKKTKNIVFTKEDTITVQKYDSAGTNLEGNAVEIKTLDELKNALK

SEQ ID NO: 172 - DNA, 822 bp, Artificial Sequence
  Synthetic nucleotide
atgaaaaaatatttattgggaataggtctaatattagccttaatagcatgtaagcaaaatgttagcagccttgatgaaaaaaatagcgtttcagtagatttacctggtggaatgaaagttcttgtaagtaaagaaaaagacaaagatggtaaatacagtctaatggcaacagtagaaaagcttgagcttaaaggaacttctgataaaaacaacggttctggaacacttgaaggtgaaaaaactgacaaaagtaaagtaaaattaacaattgctgaggatctaagtaaaaccacatttgaaatcttcaaagaagatggcaaaacattagtatcaaaaaaagtaacccttaaagacaagtcatcaacagaagaaaaattcaacgaaaagggtgaaatatctgaaaaaacaatagtaagagcaaatggaaccagacttgaatacacagacataaaaagcgataaaaccggaaaagctaaagaagttttaaaagactttactcttgaaggaactctagctgctgacggcaaaacaacattgaaagttacagaaggcactgttactttaagcaagaacatttcaaaatccggagaaataacagttgcacttgatgacactgactctagcggcaataaaaaatccggaacatgggattcagatacttctactttaacaattagtaaaaacagtcaaaaaactaaacaacttgtattcacaaaagaaaacacaataacagtacaaaactataacagagcaggcaatgcgcttgaaggcagcccagctgaaattaaagatcttgcagagcttaaagccgctttaaaataa

SEQ ID NO: 173 - protein, 273 aa, Artificial Sequence
  Synthetic peptide
MKKYLLGIGLILALIACKQNVSSLDEKNSVSVDLPGGMKVLVSKEKDKDGKYSLMATVEKLELKGTSDKNNGSGTLEGEKTDKSKVKLTIAEDLSKTTFEIFKEDGKTLVSKKVTLKDKSSTEEKFNEKGEISEKTIVRANGTRLEYTDIKSDKTGKAKEVLKDFTLEGTLAADGKTTLKVTEGTVTLSKNISKSGEITVALDDTDSSGNKKSGTWDSDTSTLTISKNSQKTKQLVFTKENTITVQNYNRAGNALEGSPAEIKDLAELKAALK